European Patent Application EP 4 684 804 A1, published January 28, 2026. Title: Conjugation product comprising an antigen binding moiety and a mucin binding moiety. Applicant: Freie Universität Berlin. The sequence listing filed with the application follows.

SEQUENCE LISTING (137 sequences)

SEQ ID NO: 1 - protein, 59 aa, Homo sapiens
EEYVGLSANQCAVPAKDRVDCGYPHVTPKECNNRGCCFDSRIPGVPWCFKPLQEAEKTF

SEQ ID NO: 2 - protein, 23 aa, Homo sapiens
EEQAKTFLDKFNHEAEDLFYQSS

SEQ ID NO: 3 - protein, 31 aa, Homo sapiens
EEQAKTFLDKFNHEAEDLFYQSSGLGKGDFR

SEQ ID NO: 4 - protein, 31 aa, Homo sapiens
  CROSSLNK 4..8: note = Side chain cyclization between lysine 4 and aspartate 8.
EEQKKTFDDKFNHEAEDLFYQSSGLGKGDFR

SEQ ID NO: 5 - protein, 31 aa, Homo sapiens
  CROSSLNK 8..12: note = Side chain cyclization between lysine 8 and aspartate 12.
EEQAKTFKDKFDHEAEDLFYQSSGLGKGDFR

SEQ ID NO: 6 - protein, 31 aa, Homo sapiens
  CROSSLNK 11..15: note = Side chain cyclization between lysine 11 and aspartate 15.
EEQAKTFLDKKNHEDEDLFYQSSGLGKGDFR

SEQ ID NO: 7 - protein, 31 aa, Homo sapiens
  CROSSLNK 15..19: note = Side chain cyclization between lysine 15 and aspartate 19.
EEQAKTFLDKFNHEKEDLDYQSSGLGKGDFR

SEQ ID NO: 8 - protein, 31 aa, Homo sapiens
  CROSSLNK 18..22: note = Side chain cyclization between lysine 18 and aspartate 22.
EEQAKTFLDKFNHEAEDKFYQDSGLGKGDFR

SEQ ID NO: 9 - protein, 31 aa, Homo sapiens
  CROSSLNK 8..12: note = Side chain cyclization between lysine 8 and aspartate 12.
  CROSSLNK 18..22: note = Side chain cyclization between lysine 18 and aspartate 22.
EEQAKTFKDKFDHEAEDKFYQDSGLGKGDFR

SEQ ID NO: 10 - protein, 31 aa, Homo sapiens
  SITE 15: note = X is an alkenylated (R)-alanine residue.
  CROSSLNK 15..22: note = Cyclization between X15 and X22 via a 7-undecenyl residue.
  SITE 22: note = X is an alkenylated (S)-alanine residue.
EEQAKTFLDKFNHEXEDLFYQXSGLGKGDFR

SEQ ID NO: 11 - protein, 31 aa, Homo sapiens
  SITE 1: note = X is N-acetylglutamate.
  SITE 15: note = X is an alkenylated (R)-alanine residue.
  CROSSLNK 15..22: note = Cyclization between X15 and X22 via a 7-undecenyl residue.
  SITE 22: note = X is an alkenylated (S)-alanine residue.
XEQAKTFLDKFNHEXEDLFYQXSGLGKGDFR

SEQ ID NO: 12 - protein, 31 aa, Homo sapiens
  SITE 18: note = X is an alkenylated (S)-alanine residue.
  CROSSLNK 18..22: note = Cyclization between X18 and X22 via a 4-octenyl residue.
  SITE 22: note = X is an alkenylated (S)-alanine residue.
EEQAKTFLDKFNHEAEDXFYQXSGLGKGDFR

SEQ ID NO: 13 - protein, 31 aa, Homo sapiens
  SITE 1: note = X is N-acetylglutamate.
  SITE 18: note = X is an alkenylated (S)-alanine residue.
  CROSSLNK 18..22: note = Cyclization between X18 and X22 via a 4-octenyl residue.
  SITE 22: note = X is an alkenylated (S)-alanine residue.
XEQAKTFLDKFNHEAEDXFYQXSGLGKGDFR

SEQ ID NO: 14 - protein, 59 aa, Homo sapiens
EEYVGLSANQCAVPAKDRVDCGYPHVTPKECNNRGCCFDSRIPGVPWCFKPLQEAECTF

SEQ ID NO: 15 - protein, 24 aa, synthetic construct
  REGION 1..24: note = Mucin binding moiety precursor
  SITE 22: note = X is azidolysine.
CCFDSRIPGVPWCFKPLQEAEXTF

SEQ ID NO: 16 - protein, 35 aa, synthetic construct
  REGION 1..35: note = Mucin binding moiety precursor
  SITE 35: note = X is a glycin residue modified with an N-acylbenzimidazole.
EEYVGLSANQCAVPAKDRVDCGYPHVTPKECNNRX

SEQ ID NO: 17 - protein, 31 aa, synthetic construct
  REGION 1..31: note = Virus binding moiety precursor
  SITE 1: note = X is a glutamte residue carrying a linker comprising two subsequent units of 8-amino-3,6-dioxaoctanoic acid, followed by a 4-pentynoic acid unit.
XEQAKTFLDKFNHEAEDLFYQSSGLGKGDFR

SEQ ID NO: 18 - protein, 88 aa, synthetic construct
  REGION 1..88: note = Peptide comprising a mucin binding moiety and a virus binding moiety
  SITE 57: note = X is a lysine residue modified at its C-terminus with a threonine-phenylalanine dipeptide. X is bound through its side chain to a 10,19-dioxo-21-(1H-1,2,3-triazol-4-yl)-3,6,12,15-tetraoxa-9,18-diazahenicosanoic acid linker. The free carboxylic acid in the linker is attached to the N-terminus of glutamate 58.
EEYVGLSANQCAVPAKDRVDCGYPHVTPKECNNRGCCFDSRIPGVPWCFKPLQEAEXEEQAKTFLDKFNHEAEDLFYQSSGLGKGDFR

SEQ ID NO: 19 - protein, 93 aa, synthetic construct
GEEYVGLSANQCAVPAKDRVDCGYPHVTPKECNNRGCCFDSRIPGVPWCFKPLQEAEATFGTEEQAKTFLDKFNHEAEDLFYQSSGLGKGDFR

SEQ ID NO: 20 - protein, 84 aa, Homo sapiens
MATMENKVICALVLVSMLALGTLAEAQTETCTVAPRERQNCGFPGVTPSQCANKGCCFDDTVRGVPWCFYPNTIDVPPEEECEF

SEQ ID NO: 21 - protein, 129 aa, Homo sapiens
MGRRDAQLLAALLVLGLCALAGSEKPSPCQCSRLSPHNRTNCGFPGITSDQCFDNGCCFDSSVTGVPWCFHPLPKQESDQCVMEVSDRRNCGYPGISPEECASRKCCFSNFIFEVPWCFFPKSVEDCHY

SEQ ID NO: 22 - protein, 217 aa, Artocarpus heterophyllus
MAYSSLLSLSVLALLFSISSADTRKWFLANGINQNPIGIIEAAVGVSEDLLNLNGMEAKNDEQSGISQTVIVGPWGAKVSTSSNGKAFDDGAFTGIREINLSYNKETAIGDFQVVYDLNGSPYVGQNHKSFITGFTPVKISLDFPSEYIMEVSGYTGNVSGYVVVRSLTFKTNKKTYGPYGVTSGTPFNLPIENGLIVGFKGSIGYWLDYFSMYLSL

SEQ ID NO: 23 - protein, 23 aa, synthetic construct
ECQAKTFLDKFNHEAEDLFYQSS

SEQ ID NO: 24 - protein, 23 aa, synthetic construct
EECAKTFLDKFNHEAEDLFYQSS

SEQ ID NO: 25 - protein, 23 aa, synthetic construct
EEQCKTFLDKFNHEAEDLFYQSS

SEQ ID NO: 26 - protein, 23 aa, synthetic construct
EEQACTFLDKFNHEAEDLFYQSS

SEQ ID NO: 27 - protein, 23 aa, synthetic construct
EEQAKCFLDKFNHEAEDLFYQSS

SEQ ID NO: 28 - protein, 23 aa, synthetic construct
EEQAKTCLDKFNHEAEDLFYQSS

SEQ ID NO: 29 - protein, 23 aa, synthetic construct
EEQAKTFCDKFNHEAEDLFYQSS

SEQ ID NO: 30 - protein, 23 aa, synthetic construct
EEQAKTFLCKFNHEAEDLFYQSS

SEQ ID NO: 31 - protein, 23 aa, synthetic construct
EEQAKTFLDCFNHEAEDLFYQSS

SEQ ID NO: 32 - protein, 23 aa, synthetic construct
EEQAKTFLDKCNHEAEDLFYQSS

SEQ ID NO: 33 - protein, 23 aa, synthetic construct
EEQAKTFLDKFCHEAEDLFYQSS

SEQ ID NO: 34 - protein, 23 aa, synthetic construct
EEQAKTFLDKFNCEAEDLFYQSS

SEQ ID NO: 35 - protein, 23 aa, synthetic construct
EEQCKTFCDKFNHEAEDLFYQSS

SEQ ID NO: 36 - protein, 23 aa, synthetic construct
EEQAKTFCDKFCHEAEDLFYQSS

SEQ ID NO: 37 - protein, 23 aa, synthetic construct
EEQAKTFLDKCNHECEDLFYQSS

SEQ ID NO: 38 - protein, 23 aa, synthetic construct
EEQAKTFLDKFNHECEDLCYQSS

SEQ ID NO: 39 - protein, 23 aa, synthetic construct
EEQAKTFLDKFNHEAEDCFYQCS

SEQ ID NO: 40 - protein, 23 aa, synthetic construct
EEQCKTFCDKFNHEAEDCFYQCS

SEQ ID NO: 41 - protein, 36 aa, synthetic construct
EAAAKEEQAKTFLDKFNHEAEDLFYQSSGLGKGDFR

SEQ ID NO: 42 - protein, 32 aa, synthetic construct
  DISULFID 23..32: note = Disulfide bridge between cysteine 23 and cysteine 32.
EEQAKTFLDKFNHEAEDLFYQSCGLGKGDFRC

SEQ ID NO: 43 - protein, 37 aa, synthetic construct
  DISULFID 28..37: note = Disulfide bridge between cysteine 28 and cysteine 37.
EAAAKEEQAKTFLDKFNHEAEDLFYQSCGLGKGDFRC

SEQ ID NO: 44 - protein, 5 aa, synthetic construct
GGGGS

SEQ ID NO: 45 - protein, 5 aa, synthetic construct
EAAAK

SEQ ID NO: 46 - protein, 11 aa, synthetic construct
GTSGSGLPSTG

SEQ ID NO: 47 - protein, 10 aa, synthetic construct
GTSYAHQAHY

SEQ ID NO: 48 - protein, 15 aa, synthetic construct
ARDFYDYDVFYYAMD

SEQ ID NO: 49 - protein, 9 aa, synthetic construct
IQIIPKSSW

SEQ ID NO: 50 - protein, 9 aa, synthetic construct
RGHFYGSGS

SEQ ID NO: 51 - protein, 10 aa, synthetic construct
IQIIPKDSWS

SEQ ID NO: 52 - protein, 9 aa, synthetic construct
PTIKKGYNN

SEQ ID NO: 53 - protein, 14 aa, synthetic construct
CARLYTKSSNANYW

SEQ ID NO: 54 - protein, 15 aa, synthetic construct
CARGGLYSSDAFDVW

SEQ ID NO: 55 - protein, 49 aa, synthetic construct
KLLGIETPLPKKELLLPGNNRKVYELSNVQEDSQPMCYSNCPDGQSTAK

SEQ ID NO: 56 - protein, 11 aa, synthetic construct
RSGNYPYAMDY

SEQ ID NO: 57 - protein, 12 aa, synthetic construct
GLPDLEWLLYPN

SEQ ID NO: 58 - protein, 12 aa, synthetic construct
SISASGSYINYA

SEQ ID NO: 59 - protein, 12 aa, synthetic construct
RDGGRELSPFEK

SEQ ID NO: 60 - protein, 12 aa, synthetic construct
SISASGSYINYA

SEQ ID NO: 61 - protein, 14 aa, synthetic construct
LVVSTTYLPHYFDN

SEQ ID NO: 62 - protein, 14 aa, synthetic construct
LVVSETYLPHYFDN

SEQ ID NO: 63 - protein, 14 aa, synthetic construct
  SITE 1: note = X is L-cyclohexylglycine
  SITE 2: note = X is cyclopropylalanine
  SITE 7: note = X is 3,5-diiodo-tyrosine
XXVSTTXLPHYFDN

SEQ ID NO: 64 - protein, 62 aa, synthetic construct
GGSEEYVGLSANQCAVPAKDRVDCGYPHVTPKECNNRGCCFDSRIPGVPWCFKPLQEAECTF

SEQ ID NO: 65 - protein, 61 aa, synthetic construct
GGEEYVGLSANQCAVPAKDRVDCGYPHVTPKECNNRGCCFDSRIPGVPWCFKPLQEAECTF

SEQ ID NO: 66 - protein, 60 aa, synthetic construct
GEEYVGLSANQCAVPAKDRVDCGYPHVTPKECNNRGCCFDSRIPGVPWCFKPLQEAECTF

SEQ ID NO: 67 - protein, 95 aa, synthetic construct
GGSEEYVGLSANQCAVPAKDRVDCGYPHVTPKECNNRGCCFDSRIPGVPWCFKPLQEAECTFGTEEQAKTFLDKFNHEAEDLFYQSSGLGKGDFR

SEQ ID NO: 68 - protein, 94 aa, synthetic construct
GGEEYVGLSANQCAVPAKDRVDCGYPHVTPKECNNRGCCFDSRIPGVPWCFKPLQEAECTFGTEEQAKTFLDKFNHEAEDLFYQSSGLGKGDFR

SEQ ID NO: 69 - protein, 93 aa, synthetic construct
GEEYVGLSANQCAVPAKDRVDCGYPHVTPKECNNRGCCFDSRIPGVPWCFKPLQEAECTFGTEEQAKTFLDKFNHEAEDLFYQSSGLGKGDFR

SEQ ID NO: 70 - protein, 92 aa, synthetic construct
EEYVGLSANQCAVPAKDRVDCGYPHVTPKECNNRGCCFDSRIPGVPWCFKPLQEAECTFGTEEQAKTFLDKFNHEAEDLFYQSSGLGKGDFR

SEQ ID NO: 71 - protein, 150 aa, Musa acuminata
MNGAIKVGAWGGNGGSAFDMGPAYRIISVKIFSGDVVDGVDVTFTYYGKTETRHYGGSGGTPHEIVLQEGEYLVGMAGEVANYHGAVVLGKLGFSTNKKAYGPFGNTGGTPFSLPIAAGKISGFFGRGGKFLDAIGVYLEPASGENLYFQ

SEQ ID NO: 72 - protein, 143 aa, Musa acuminata
MNGAIKVGAWGGNGGSAFDMGPAYRIISVKIFSGDVVDGVDVTFTYYGKTETRHYGGSGGTPHEIVLQEGEYLVGMAGEVANYHGAVVLGKLGFSTNKKAYGPFGNTGGTPFSLPIAAGKISGFFGRGGKFLDAIGVYLEPLE

SEQ ID NO: 73 - protein, 143 aa, Musa acuminata; identical to SEQ ID NO: 72

SEQ ID NO: 74 - protein, 143 aa, Musa acuminata
MNGAIKVGAWGGNGGSAFDMGPAYRIISVKIFSGDVVDGVDVTFTYYGKTETRHYGGSGGTPHEIVLQEGEYLVGMAGEVANYTGAVVLGKLGFSTNKKAYGPFGNTGGTPFSLPIAAGKISGFFGRGGKFLDAIGVYLEPLE

SEQ ID NO: 75 - protein, 143 aa, Musa acuminata
MNGAIKVGAWGGNGGSAFDMGPAYRIISVKIFSGDVVDGVDVTFTYYGKTETRHYGGSGGTPHEIVLQEGEYLVGMAGEVANYTGAVVLGKLGFSTNKKAYGPFGNTGGTPFSLPIAAGKISGFFGRGGKFLDAIGVYLEPLA

SEQ ID NO: 76 - protein, 155 aa, Homo sapiens
ERLCHPCPWEWTFFQGNCYFMSNSQRNWHDSITACKEVGAQLVVIKSAEEQNFLQLQSSRSNRFTWMGLSDLNQEGTWQWVDGSPLLPSFKQYWNRGEPNNVGEEDCAEFSGNGWNDDKCNLAKFWICKKSAASCSRDEEQFLSPAPATPNPPPA

SEQ ID NO: 77 - protein, 147 aa, Homo sapiens
MGSERTCCPVNWVEHERSCYWFSRSGKAWADADNYCRLEDAHLVVVTSWEEQKFVQHHIGPVNTWMGLHDQNGPWKWVDGTDYETGFKNWRPEQPDDWYGHGLGGGEDCAHFTDDGRWNDDVCQRPYRWVCETELDKASQEPPLLGS

SEQ ID NO: 78 - protein, 147 aa, Homo sapiens
ALTCVMEGKDIEDWSCCPTPWTSFQSSCYFISTGMQSWTKSQKNCSVMGADLVVINTREEQDFIIQNLKRNSSYFLGLSDPGGRRHWQWVDQTPYNENVTFWHSGEPNNLDERCAIINFRSSEEWGWNDIHCHVPQKSICKMKKIYI

SEQ ID NO: 79 - protein, 117 aa, Homo sapiens
TCRYLLVRSLQTFSQAWFTCRRCYRGNLVSIHNFNINYRIQCSVSALNQGQVWIGGRITGSGRCRRFQWVDGSRWNFAYWAAHQPWSRGGHCVALCTRGGYWRRAHCLRRLPFICSY

SEQ ID NO: 80 - protein, 155 aa, Homo sapiens
SQLRKAIGEMDNQVSQLTSELKFIKNAVAGVRETESKIYLLVKEEKRYADAQLSCQGRGGTLSMPKDEAANGLMAAYLAQAGLARVFIGINDLEKEGAFVYSDHSPMRTFNKWRSGEPNNAYDEEDCVEMVASGGWNDVACHTTMYFMCEFDKEN

SEQ ID NO: 81 - protein, 155 aa, Homo sapiens; identical to SEQ ID NO: 76

SEQ ID NO: 82 - protein, 139 aa, Homo sapiens
AERLCRHCPKDWTFFQGNCYFMSNSQRNWHDSVTACQEVRAQLVVIKTAEEQNFLQLQTSRSNRFSWMGLSDLNQEGTWQWVDGSPLSPSFQRYWNSGEPNNSGNEDCAEFSGSGWNDNRCDVDNYWICKKPAACFRDE

SEQ ID NO: 83 - protein, 134 aa, Homo sapiens
GSCPKNWKSFSSNCYFISTESASWQDSEKDCARMEAHLLVINTQEEQDFIFQNLQEESAYFVGLSDPEGQRHWQWVDQTPYNESSTFWHPREPSDPNERCVVLNFRKSPKRWGWNDVNCLGPQRSVCEMMKIHL

SEQ ID NO: 84 - protein, 147 aa, Homo sapiens
ALTCFSEGTKVPAWGCCPASWKSFGSSCYFISSEEKVWSKSEQNCVEMGAHLVVFNTEAEQNFIVQQLNESFSYFLGLSDPQGNNNWQWIDKTPYEKNVRFWHLGEPNHSAEQCASIVFWKPTGWGWNDVICETRRNSICEMNKIYL

SEQ ID NO: 85 - protein, 157 aa, Homo sapiens
WSYNTSTEAMTYDEASAYCQQRYTHLVAIQNKEEIEYLNSILSYSPSYYWIGIRKVNNVWVWVGTQKPLTEEAKNWAPGEPNNRQKDEDCVEIYIKREKDVGMWNDERCSKKKLALCYTAACTNTSCSGHGECVETINNYTCKCDPGFSGLKCEQIV

SEQ ID NO: 86 - protein, 482 aa, Homo sapiens
APLADAALPEPNVFLIFSHGLQGCLEAQGGQVRVTPACNTSLPAQRWKWVSRNRLFNLGTMQCLGTGWPGTNTTASLGMYECDREALNLRWHCRTLGDQLSLLLGARTSNISKPGTLERGDQTRSGQWRIYGSEEDLCALPYHEVYTIQGNSHGKPCTIPFKYDNQWFHGCTSTGREDGHLWCATTQDYGKDERWGFCPIKSNDCETFWDKDQLTDSCYQFNFQSTLSWREAWASCEQQGADLLSITEIHEQTYINGLLTGYSSTLWIGLNDLDTSGGWQWSDNSPLKYLNWESDQPDNPSEENCGVIRTESSGGWQNRDCSIALPYVCKKKPNATAEPTPPDRWANVKVECEPSWQPFQGHCYRLQAEKRSWQESKKACLRGGGDLVSIHSMAELEFITKQIKQEVEELWIGLNDLKLQMNFEWSDGSLVSFTHWHPFEPNNFRDSLEDCVTIWGPEGRWNDSPCNQSLPSICKKAGQLSG

SEQ ID NO: 87 - protein, 149 aa, Homo sapiens
EEPQRELPSARIRCPKGSKAYGSHCYALFLSPKSWTDADLACQKRPSGNLVSVLSGAEGSFVSSLVKSIGNSYSYVWIGLHDPTQGTEPNGEGWEWSSSDVMNYFAWERNPSTISSPGHCASLSRSTAFLRWKDYNCNVRLPYVCKFTD

SEQ ID NO: 88 - protein, 140 aa, Homo sapiens
ETGGLLNCPIYWQQLREKCLLFSHTVNPWNNSLADCSTKESSLLLIRDKDELIHTQNLIRDKAILFWIGLNFSLSEKNWKWINGSFLNSNDLEIRGDAKENSCISISQTSVYSEYCSTEIRWICQKELTPVRNKVYPDSK

SEQ ID NO: 89 - protein, 164 aa, Homo sapiens
WTYHYSEKPMNWQRARRFCRDNYTDLVAIQNKAEIEYLEKTLPFSRSYYWIGIRKIGGIWTWVGTNKSLTEEAENWGDGEPNNKKNKEDCVEIYIKRNKDAGKWNDDACHKLKAALCYTASCQPWSCSGHGECVEIINNYTCNCDVGYYGPQCQFVQVDPRLID

SEQ ID NO: 90 - protein, 146 aa, Homo sapiens
QVVSQGWKYFKGNFYYFSLIPKTWYSAEQFCVSRNSHLTSVTSESEQEFLYKTAGGLIYWIGLTKAGMEGDWSWVDDTPFNKVQSVRFWIPGEPNNAGNNEHCGNIKAPSLQAWNDAPCDKTFLFICKRPYVPSEPSAWSHPQFEK

SEQ ID NO: 91 - protein, 115 aa, Homo sapiens
NVGKKYFMSSVRRMPLNRAKALCSELQGTVATPRNAEENRAIQNVAKDVAFLGITDQRTENVFEDLTGNRVRYTNWNEGEPNNVGSGENCVVLLTNGKWNDVPCSDSFLVVCEFS

SEQ ID NO: 92 - protein, 147 aa, Homo sapiens
MGSVKNCCPLNWEYFQSSCYFFSTDTKSWALSLKNCSAMGAHLVVINSQEEQEFLSYKKPKMREFFIGLSDQVVEGQWQWVDGTPLTKSLSFWDVGEPNNIATLEDCATMRDSSNPRQNWNDVTCFLNYFRICEMVGINPLNKGKSL

SEQ ID NO: 93 - protein, 162 aa, Homo sapiens
WTYHYSTKAYSWNISRKYCQNRYTDLVAIQNKNEIDYLNKVLPYYSSYYWIGIRKNNKTWTWVGTKKALTNEAENWADNEPNNKRNNEDCVEIYIKSPSAPGKWNDEHCLKKKHALCYTASCQDMSCSKQGECLETIGNYTCSCYPGFYGPECEYVRDDDDK

SEQ ID NO: 94 - protein, 131 aa, Homo sapiens
QSCAPGWFYHKSNCYGYFRKLRNWSDAELECQSYGNGAHLASILSLKEASTIAEYISGYQRSQSIWIGLHDPQKRQQWQWIDGAMYLYRSWSGKSMGGNKHCAEMSSNNNFLTWSSNECNKRQHFLCKYRP

SEQ ID NO: 95 - protein, 158 aa, Homo sapiens
EAEAGSVASLRQQVEALQGQVQHLQAAFSQYKKVELFPNGQSVGEKIFKTAGFVKPFTEAQLLCTQAGGQLASPRSAAENAALQQLVVAKNEAAFLSMTDSKTEGKFTYPTGESLVYSNWAPGEPNDDGGSEDCVEIFTNGKWNDRACGEKRLVVCEF

SEQ ID NO: 96 - protein, 140 aa, Homo sapiens
EDNSCPPHWKNFTDKCYYFSVEKEIFEDAKLFCEDKSSHLVFINTREEQQWIKKQMVGRESHWIGLTDSERENEWKWLDGTSPDYKNWKAGQPDNWGHGHGPGEDCAGLIYAGQWNDFQCEDVNNFICEKDRETVLSSAL

SEQ ID NO: 97 - protein, 182 aa, Homo sapiens
GEPPTQKPKKIVNAKKDVVNTKMFEELKSRLDTLSQEVALLKEQQALQTVCLKGTKVHMKCFLAFTQTKTFHEASEDCISRGGTLSTPQTGSENDALYEYLRQSVGNEAEIWLGLNDMAAEGTWVDMTGARIAYKNWETEITAQPDGGKTENCAVLSGAANGKWFDKRCRDQLPYICQFGIV

SEQ ID NO: 98 - protein, 127 aa, Homo sapiens
GQKSNRKDYSLTMQSSVTVQEGMCVHVRCSFSYPVDSQTDSDPVHGYWFRAGNDISWKAPVATNNPAWAVQEETRDRFHLLGDPQTKNCTLSIRDARMSDAGRYFFRMEKGNIKWNYKYDQLSVNVT

SEQ ID NO: 99 - protein, 116 aa, Homo sapiens
GSPGTPEVKVASSEDVDLPCTAPWDPQVPYTVSWVKLLEGGEERMETPQEDHLRGQHYHQKGQNGSFDAPNERPYSLKIRNTTSSNSGTYRCTLQDPDGQRNLSGKVILRVTGSPA

SEQ ID NO: 100 - protein, 318 aa, Homo sapiens
ETGDSSKWVFEHPETLYAWEGACVWIPCTYRALDGDLESFILFHNPEYNKATSKFDGTRLYESTKDGKVPSEQKRVQFLGDKNKNCTLSIHPVHLADSGQLGLRMESKTEKWMERIHLAVSERPFPPHIQLPPEIQESQEVTLTCLLAFSCYGYPIQLQWLLEGVPMRQAAVTSTSLTIKSVFTRSELKFSPQWSHHGKIVTCQLQDADGKFLSADTVQLNVKHTPKLEIKVTPSDAIVREGDSVTMTCEVSSSNPEYTTVSWLKDGTSLKKQNTFTLNLREVTKDQSGKYCCQVSNDVGPGRSEEVFLQVQYAGGTK

SEQ ID NO: 101 - protein, 127 aa, Homo sapiens
GDPNFWLQVQESVTVQEGLCVLVPCTFFHPIPYYDKNSPVHGYWFREGAIISRDSPVATNKLDQEVQEETQGRFRLLGDPSRNNCSLSIVDARRRDNGSYFFRMERGSTKYSYKSPQLSVHVTDLTH

SEQ ID NO: 102 - protein, 127 aa, Homo sapiens; identical to SEQ ID NO: 98

SEQ ID NO: 103 - protein, 127 aa, Homo sapiens; identical to SEQ ID NO: 98

SEQ ID NO: 104 - protein, 145 aa, Homo sapiens
MEGDRQYGDGYLLQVQELVTVQEGLSVHVPCSFSYPQDGWTDSDPVHGYWFRAGDRPYQDAPVATNNPDREVQAETQGRFQLLGDIWSNDCSLSIRDARKRDKGSYFFRLERGSMKWSYKSQLNYKTKQLSVFVTALTHGSLVPR

SEQ ID NO: 105 - protein, 309 aa, Homo sapiens
FVRTKIDTTENLLNTEVHSSPAQRWSMQVPPEVSAEAGDAAVLPCTFTHPHRHYDGPLTAIWRAGEPYAGPQVFRCAAARGSELCQTALSLHGRFRLLGNPRRNDLSLRVERLALADDRRYFCRVEFAGDVHDRYESRHGVRLHVTAAPRIVNISVLPSPAHAFRALCTAEGEPPPALAWSGPALGNSLAAVRSPREGHGHLVTAELPALTHDGRYTCTAANSLGRSEASVYLFRFHGASGASTVALLLGALGFKALLLLGVLAARAARRRPEHLDTPDTPPRSQAQESNYENLSQMNPRSPPATMCSP

SEQ ID NO: 106 - protein, 137 aa, Homo sapiens
LIVPYNLPLPGGVVPRMLITILGTVKPNANRIALDFQRGNDVAFHFNPRFNENNRRVIVCNTKLDNNWGREERQSVFPFESGKPFKIQVLVEPDHFKVAVNDAHLLQYNHRVKKLNEISKLGISGDIDLTSASYTMI

SEQ ID NO: 107 - protein, 134 aa, Homo sapiens
ACGLVASNLNLKPGECLRVRGEVAPDAKSFVLNLGKDSNNLCLHFNPRFNAHGDANTIVCNSKDGGAWGTEQREAVFPFQPGSVAEVCITFDQANLTVKLPDGYEFKFPNRLNLEAINYMAADGDFKIKCVAFD

SEQ ID NO: 108 - protein, 135 aa, Homo sapiens
GSHMTGELEVKNMDMKPGSTLKITGSIADGTDGFVINLGQGTDKLNLHFNPRFSESTIVCNSLDGSNWGQEQREDHLCFSPGSEVKFTVTFESDKFKVKLPDGHELTFPNRLGHSHLSYLSVRGGFNMSSFKLKE

SEQ ID NO: 109 - protein, 146 aa, Homo sapiens
GPYGAPAGPLIVPYNLPLPGGVVPRMLITILGTVKPNANRIALDFQRGNDVAFHFNPRFNENNRRVIVCNTKLDNNWGREERQSVFPFESGKPFKIQVLVEPDHFKVAVNDAHLLQYNHRVKKLNEISKLGISGDIDLTSASYTMI

SEQ ID NO: 110 - protein, 153 aa, Homo sapiens
HCHQQLNSLPTMEGPPTFNPPVPYFGRLQGGLTARRTIIIKGYVPPTGKSFAINFKVGSSGDIALHINPRMGNGTVVRNSLLNGSWGSEEKKITHNPFGPGQFFDLSIRCGLDRFKVYANGQHLFDFAHRLSAFQRVDTLEIQGDVTLSYVQI

SEQ ID NO: 111 - protein, 154 aa, Homo sapiens
MMLSLNNLQNIIYNPVIPFVGTIPDQLDPGTLIVIRGHVPSDADRFQVDLQNGSSVKPRADVAFHFNPRFKRAGCIVCNTLINEKWGREEITYDTPFKREKSFEIVIMVLKDKFQVAVNGKHTLLYGHRIGPEKIDTLGIYGKVNIHSIGFSFS

SEQ ID NO: 112 - protein, 148 aa, Homo sapiens
MAFSGSQAPYLSPAVPFSGTIQGGLQDGLQITVNGTVLSSSGTRFAVNFQTGFSGNDIAFHFNPRFEDGGYVVCNTRQNGSWGPEERKTHMPFQKGMPFDLCFLVQSSDFKVMVNGILFVQYFHRVPFHRVDTISVNGSVQLSYISFQ

SEQ ID NO: 113 - protein, 142 aa, Homo sapiens
GSHMSSLPVPYKLPVSLSVGSCVIIKGTPIHSFINDPQLQVDFYTDMDEDSDIAFRFRVHFGNHVVMNRREFGIWMLEETTDYVPFEDGKQFELCIYVHYNEYEIKVNGIRIYGFVHRIPPSFVKMVQVSRDISLTSVSVCN

SEQ ID NO: 114 - protein, 218 aa, Homo sapiens
QSCATGPRNCKDLLDRGHFLSGWHTIYLPDCRPLTVLCDMDTDGGGWTVFQRRMDGSVDFYRDWAAYKQGFGSQLGEFWLGNDNIHALTAQGSSELRTDLVDFEGNHQFAKYKSFKVADEAEKYKLVLGAFVGGSAGNSLTGHNNNFFSTKDQDNDVSSSNCAEKFQGAWWYADCHASNLNGLYLMGPHESYANGINWSAAKGYKYSYKVSEMKVRPA

SEQ ID NO: 115 - protein, 226 aa, Homo sapiens
ATGSRPRDCLDVLLSGQQDDGVYSVFPTHYPAGFQVYCDMRTDGGGWTVFQRREDGSVNFFRGWDAYRDGFGRLTGEHWLGLKRIHALTTQAAYELHVDLEDFENGTAYARYGSFGVGLFSVDPEEDGYPLTVADYSGTAGDSLLKHSGMRFTTKDRDSDHSENNCAAFYRGAWWYRNCHTSNLNGQYLRGAHASYADGVEWSSWTGWQYSLKFSEMKIRPVREDR

SEQ ID NO: 116 - protein, 221 aa, Homo sapiens
DLVNLLRCQEGPRNCRELLSQGATLSGWYHLCLPEGRALPVFCDMDTEGGGWLVFQRRQDGSVDFFRSWSSYRAGFGNQESEFWLGNENLHQLTLQGNWELRVELEDFNGNRTFAHYATFRLLGEVDHYQLALGKFSEGTAGDSLSLHSGRPFTTYDADHDSSNSNCAVIVHGAWWYASCYRSNLNGRYAVSEAAAHKYGIDWASGRGVGHPYRRVRMMLR

SEQ ID NO: 117 - protein, 306 aa, Homo sapiens
TDWSHPQFEKSTDEANTYFKEWTCSSSPSLPRSCKEIKDECPSAFDGLYFLRTENGVIYQTFCDMTSGGGGWTLVASVHENDMRGKCTVGDRWSSQQGSKAVYPEGDGNWANYNTFGSAEAATSDDYKNPGYYDIQAKDLGIWHVPNKSPMQHWRNSSLLRYRTDTGFLQTLGHNLFGIYQKYPVKYGEGKCWTDNGPVIPVVYDFGDAQKTASYYSPYGQREFTAGFVQFRVFNNERAANALCAGMRVTGCNTEHHCIGGGGYFPEASPQQCGDFSGFDWSGYGTHVGYSSSREITEAAVLLFYR

SEQ ID NO: 118 - protein, 218 aa, Homo sapiens
NPCLTGPRTCKDLLDRGHFLSGWHTIYLPDCRPLTVLCDMDTDGGGWTVFQRRVDGSVDFYRDWATYKQGFGSRLGEFWLGNDNIHALTAQGTSELRTDLVDFEDNYQFAKYRSFKVADEAEKYNLVLGAFVEGSAGDSLTFHNNQSFSTKDQDNDLNTGNCAVMFQGAWWYKNCHTSNLNGRYLRGTHGSFANGINWKSGKGYNYSYKVSEMKVRPA

SEQ ID NO: 119 - protein, 217 aa, Homo sapiens
SCATGPRNCKDLLDRGYFLSGWHTIYLPDCRPLTVLCDMDTDGGGWTVFQRRMDGSVDFYRDWAAYKQGFGSQLGEFWLGNDNIHALTAQGSSELRVDLVDFEGNHQFAKYKSFKVADEAEKYKLVLGAFVGGSAGNSLTGHNNNFFSTKDQDNDVSSSNCAEKFQGAWWYADCHASNLNGLYLMGPHESFANGINWSAAKGYKYSYKVSEMKVRPA

SEQ ID NO: 120 - protein, 17 aa, Homo sapiens
AGTTPSPVPTTSTTSAA

SEQ ID NO: 121 - protein, 516 aa, Clostridium thermocellum
SSGLVPRGSHMASMTGGQQMGRGSEFAAEGVIVNGTQFKDTSGNVIHAHGGGMLKHGDYYYWYGEYRDDSNLFLGVSCYRSKDLVNWEYRGEVLSRNSAPELNHCNIERPKVMYNASTGEFVMWMHWENGINYGQARAAVAYSKTPDGKFTYIRSFRPMQDTGVMDHGLPGYMSRDCNVFVDTDGKGYFISAANENMDLHLYELTPDYKNIASLKAKLFVGQQREAPCLIKRNGYYYLITSGCTGWNPNQAKYAYSKDLASGWSQLYNLGNSTTYRSQPTFIIPVQGSSGTSYLYMGDRWAGAWGGKVNDSQYVWLPLNFISDTTLELPYYDSVKIDASSGIISEYIPDTTRYKLVNKNSGKVLDVLDGSVDNAAQIVQWTDNGSLSQQWYLVDVGGGYKKIVNVKSGRALDVKDESKEDGGVLIQYTSNGGYNQHWKFTDIGDGYYKISSRHCGKLIDVRKWSTEDGGIIQQWSDAGGTNQHWKLVLVSSPEPSPSPSPQVVKGDVNGDLKVNST

SEQ ID NO: 122 - protein, 371 aa, Homo sapiens
AMADIGSYKLVCYFTNWSQDRQEPGKFTPENIDPFLCSHLIYSFASIENNKVIIKDKSEVMLYQTINSLKTKNPKLKILLSIGGYLFGSKGFHPMVDSSTSRLEFINSIILFLRNHNFDGLDVSWIYPDQKENTHFTVLIHELAEAFQKDFTKSTKERLLLTVGVSAGRQMIDNSYQVEKLAKDLDFINLLSFDFHGSWEKPLITGHNSPLSKGWQDRGPSSYYNVEYAVGYWIHKGMPSEKVVMGIPTYGHSFTLASAETTVGAPASGPGAAGPITESSGFLAYYEICQFLKGAKITWLQDQQVPYAVKGNQWVGYDDVKSMETKVQFLKNLNLGGAMIWSIDMDDFTGKSCNQGPYPLVQAVKRSLGSL

SEQ ID NO: 123 - protein, 365 aa, Homo sapiens
AYKLVCYFTNWSQDRQEPGKFTPENIDPFLCSHLIYSFASIENNKVIIKDKSEVMLYQTINSLKTKNPKLKILLSIGGYLFGSKGFHPMVDSSTSRLEFINSIILFLRNHNFDGLDVSWIYPDQKENTHFTVLIHELAEAFQKDFTKSTKERLLLTAGVSAGRQMIDNSYQVEKLAKDLDFINLLSFDFHGSWEKPLITGHNSPLSKGWQDRGPSSYYNVEYAVGYWIHKGMPSEKVVMGIPTYGHSFTLASAETTVGAPASGPGAAGPITESSGFLAYYEICQFLKGAKITRLQDQQVPYAVKGNQWVGYDDVKSMETKVQFLKNLNLGGAMIWSIDMDDFTGKSCNQGPYPLVQAVKRSLGSL

SEQ ID NO: 124 - protein, 362 aa, Homo sapiens [sequence omitted]

SEQ ID NO: 125 - protein, 393 aa, Homo sapiens
MRTLFNLLWLALACSPVHTTLSKSDAKKAASKTLLEKSQFSDKPVQDRGLVVTDLKAESVVLEHRSYCSAKARDRHFAGDVLGYVTPWNSHGYDVTKVFGSKFTQISPVWLQLKRRGREMFEVTGLHDVDQGWMRAVRKHAKGLHIVPRLLFEDWTYDDFRNVLDSEDEIEELSKTVVQVAKNQHFDGFVVEVWNQLLSQKRVGLIHMLTHLAEALHQARLLALLVIPPAITPGTDQLGMFTHKEFEQLAPVLDGFSLMTYDYSTAHQPGPNAPLSWVRACVQVLDPKSKWRSKILLGLNFYGMDYATSKDAREPVVGARYIQTLKDHRPRMVWDSQASEHFFEYKKSRSGRHVVFYPTLKSLQVRLELARELGVGVSIWELGQGLDYFYDLL

SEQ ID NO: 126 - protein, 204 aa, Homo sapiens
HTDLSGKVFVFPRESVTDHVNLITPLEKPLQNFTLCFRAYSDLSRAYSLFSYNTQGRDNELLVYKERVGEYSLYIGRHKVTSKVIEKFPAPVHICVSWESSSGIAEFWINGTPLVKKGLRQGYFVEAQPKIVLGQEQDSYGGKFDRSQSFVGEIGDLYMWDSVLPPENILSAYQGTPLPANILDWQALNYEIRGYVIIKPLVWV

SEQ ID NO: 127 - protein, 265 aa, Homo sapiens
NKGSIEGREPAVYFKEQFLDGDGWTSRWIESKHKSDFGKFVLSSGKFYGDEEKDKGLQTSQDARFYALSASFEPFSNKGQTLVVQFTVKHEQNIDCGGGYVKLFPNSLDQTDMHGDSEYNIMFGPDICGPGTKKVHVIFNYKGKNVLINKDIRCKDDEFTHLYTLIVRPDNTYEVKIDNSQVESGSLEDDWDFLPGSGDPSIYAYDNFGVLGLDLWQVKSGTIFDNFLITNDEAYAEEFGNETWGVTKAAEKQMKDKQDEEQRLK

SEQ ID NO: 128 - protein, 248 aa, Homo sapiens
LVPRGSHMDGVGGDPAVALPHRRFEYKYSFKGPHLVQSDGTVPFWAHAGNAIPSSDQIRVAPSLKSQRGSVWTKTKAAFENWEVEVTFRVTGRGRIGADGLAIWYAENQGLEGPVFGSADLWNGVGIFFDSFDNDGKKNNPAIVIIGNNGQIHYDHQNDGASQALASCQRDFRNKPYPVRAKITYYQNTLTVMINNGFTPDKNDYEFCAKVENMIIPAQGHFGISAATGGLADDHDVLSFLTFQLTEP

SEQ ID NO: 129 - protein, 296 aa, Homo sapiens
ETGASVEGDNCEVKDPRHGNLYDLKPLGLNDTIVSAGEYTYYFRVCGKLSSDVCPTSDKSKVVSSCQEKREPQGFHKVAGLLTQKLTYENGLLKMNFTGGDTCHKVYQRSTAIFFYCDRGTQRPVFLKETSDCSYLFEWRTQYACPPFDLTECSFKDGAGNSFDLSSLSRYSDNWEAITGTGDPEHYLINVCKSLAPQAGTEPCPPEAAACLLGGSKPVNLGRVRDGPQWRDGIIVLKYVDGDLCPDGIRKKSTTIRFTCSESQVNSRPMFISAVEDCEYTFAWPTATACPMKSTR

SEQ ID NO: 130 - protein, 124 aa, Homo sapiens
GSAPCLLKTKDWWTYEFCYGRHIQQYHMEDSEIKGEVLYLGYYQSAFDWDDETAKASKQHRLKRYHSQTYGNGSKCDLNGRPREAEVRFLCDEGAGISGDYIDRVDEPLSCSYVLTIRTPRLCP

SEQ ID NO: 131 - protein, 393 aa, Mus musculus
APLAVPTPAFPFPAPTMVHGPCVAESEPALLTGSKQFGLSRNSHIAIAFDDTKVKNRLTIELEVRTEAESGLLFYMARINHADFATVQLRNGFPYFSYDLGSGDTSTMIPTKINDGQWHKIKIVRVKQEGILYVDDASSQTISPKKADILDVVGILYVGGLPINYTTRRIGPVTYSLDGCVRNLHMEQAPVDLDQPTSSFHVGTCFANAESGTYFDGTGFAKAVGGFKVGLDLLVEFEFRTTRPTGVLLGVSSQKMDGMGIEMIDEKLMFHVDNGAGRFTAIYDAEIPGHMCNGQWHKVTAKKIKNRLELVVDGNQVDAQSPNSASTSADTNDPVFVGGFPGGLNQFGLTTNIRFRGCIRSLKLTKGTGKPLEVNFAKALELRGVQPVSCPTT

SEQ ID NO: 132 - protein, 469 aa, Homo sapiens
TRQFLIYNEDHKRCVDAVSPSAVQTAACNQDAESQKFRWVSESQIMSVAFKLCLGVPSKTDWVAITLYACDSKSEFQKWECKNDTLLGIKGEDLFFNYGNRQEKNIMLYKGSGLWSRWKIYGTTDNLCSRGYEAMYTLLGNANGATCAFPFKFENKWYADCTSAGRSDGWLWCGTTTDYDTDKLFGYCPLKFEGSESLWNKDPLTSVSYQINSKSALTWHQARKSCQQQNAELLSITEIHEQTYLTGLTSSLTSGLWIGLNSLSFNSGWQWSDRSPFRYLNWLPGSPSAEPGKSCVSLNPGKNAKWENLECVQKLGYICKKGNTTLNSFVIPSESDVPTHCPSQWWPYAGHCYKIHRDEKKIQRDALTTCRKEGGDLTSIHTIEELDFIISQLGYEPNDELWIGLNDIKIQMYFEWSDGTPVTFTKWLRGEPSHENNRQEDCVVMKGKDGYWADRGCEWPLGYICKMKS

SEQ ID NO: 133 - protein, 197 aa, Mus musculus
GSHMGSADEERDHWQQFYFLSKRRRNLLRNPCGEEDLEGWSDVEHGGDGWKVEELPGDNGVEFTQDDSVKKYFASSFEWCRKAQVIDLQAEGYWEELLDTTQPAIVVKDWYSGRTDAGSLYELTVRLLSENEDVLAEFATGQVAVPEDGSWMEISHTFIDYGPGVRFVRFEHGGQDSVYWKGWFGARVTNSSVWVEP

SEQ ID NO: 134 - protein, 190 aa, Xenopus laevis
GAMSGLADKVIWAVNAGGESHVDVHGIHYRKDPLEGRVGRASDYGMKLPILRSNPEDQVLYQTERYNEDSFGYDIPIKEEGEYVLVLKFAEVYFAQSQQKVFDVRVNGHTVVKDLDIFDRVGHSTAHDEIIPISIKKGKLSVQGEVSTFTGKLSVEFVKGYYDNPKVCALFIMKGTADDVPMLQPHPGLE

SEQ ID NO: 135 - protein, 186 aa, Triticum aestivum
QRCGEQGSGMECPNNLCCSQYGYCGMGGDYCGKGCQNGACWTSKRCGSQAGGKTCPNNHCCSQYGHCGFGAEYCGAGCQGGPCRADIKCGSQAGGKLCPNNLCCSQWGYCGLGSEFCGEGCQNGACSTDKPCGKDAGGRVCTNNYCCSKWGSCGIGPGYCGAGCQSGGCDGVFAEAIATNSTLLAE

SEQ ID NO: 136 - protein, 171 aa, Triticum aestivum
QRCGEQGSNMECPNNLCCSQYGYCGMGGDYCGKGCQNGACWTSKRCGSQAGGATCTNNQCCSQYGYCGFGAEYCGAGCQGGPCRADIKCGSQAGGKLCPNNLCCSQWGFCGLGSEFCGGGCQSGACSTDKPCGKDAGGRVCTNNYCCSKWGSCGIGPGYCGAGCQSGGCDG

SEQ ID NO: 137 - protein, 258 aa, Sambucus nigra
TSFTRNIVGRDGLCVDVRNGYDTDGTPLQLWPCGTQRNQRWTFDSDDTIRSMGKCMTANGLNNGSNIVIFNCSTAAENAIKWEVPIDGSIINPSSGLVMTAPRAASRTILLLEDNIYAASQGWTVTNNVKPIVASIVGYKEMCLQSNGENNGVWMEDCEATSLQQQWALYGDRTIRVNSTRGLCVTTNGYNSKDLIIILKCQGLPSQRWFFNSDGAIVNPKSRLVMDVRASNVSLREIIIFPATGNPNQQWVTQVLPS